European Patent Application EP 4 421 085 A1, published August 28, 2024. Title: Alpha synuclein-binding polypeptide. Applicant: Amylonix AB. The sequence listing filed with the application follows.

SEQUENCE LISTING (57 sequences)

SEQ ID NO: 1 - protein, 43 aa, synthetic construct
GGERIVLPNLNADQLCAFIRSLEDDPSQSANLVAEAKKLNDAQ

SEQ ID NO: 2 - protein, 43 aa, synthetic construct
GGERIYLPNLNADQLCAFIRSLEDDPSQSANLLAEAKKLNDAQ

SEQ ID NO: 3 - protein, 43 aa, synthetic construct
GGEPVYLPNLNADQLCAFIRSLEDDPSQSANLLAEAKKLNDAQ

SEQ ID NO: 4 - protein, 43 aa, synthetic construct
GGELVYLPNLNADQLCAFIRSAEDDPSQSANLLAEAKKLNDAQ

SEQ ID NO: 5 - protein, 43 aa, synthetic construct
GGERVYMPNLKADQLCAFIRSAEDDPSQSANLLAEAKKLNDAQ

SEQ ID NO: 6 - protein, 43 aa, synthetic construct
GGETFSLPNLNADQLCAFIRSLEDDPSQSANLVAEAKKLNDAQ

SEQ ID NO: 7 - protein, 7 aa, synthetic construct
NADQLCA

SEQ ID NO: 8 - protein, 43 aa, synthetic construct
GGERFYLPNLNPDQLCAFIRSLEDDPSQSANLIAEAKKLNDAQ

SEQ ID NO: 9 - protein, 43 aa, synthetic construct
GGERFTLPNLNADQLCAFIRSLEDDPSQSANLLAEAKKLNDAQ

SEQ ID NO: 10 - protein, 43 aa, synthetic construct
GGERFTLPNLNPDQICAFIRSVEDDPSQSANLLAEAKKLNDAQ

SEQ ID NO: 11 - protein, 43 aa, synthetic construct
GGEEVYLPNLKADQLCAFIRSVEDDPSQSANLLAEAKKLNDAQ

SEQ ID NO: 12 - protein, 43 aa, synthetic construct
GGEPVYLPNLNPDQWCAFLRSLEDDPSQSANLLAEAKKLNDAQ

SEQ ID NO: 13 - protein, 43 aa, synthetic construct
GGEPVYLPNLNADQWCAFWRSLEDDPSQSANLLAEAKKLNDAQ

SEQ ID NO: 14 - protein, 43 aa, synthetic construct
GGERVYYPNLNADQWCAFWRSLEDDPSQSANLLAEAKKLNDAQ

SEQ ID NO: 15 - protein, 43 aa, synthetic construct
GGETVLLPNLNPDQWCAFWRSLEDDPSQSANLLAEAKKLNDAQ

SEQ ID NO: 16 - protein, 43 aa, synthetic construct
GGEIVWLPNLNPDQWCAFFRSLEDDPSQSANLLAEAKKLNDAQ

SEQ ID NO: 17 - protein, 43 aa, synthetic construct
GGERVYLPNLKADQLCAFFRSLEDDPSQSANLLAEAKKLNDAQ

SEQ ID NO: 18 - protein, 10 aa, synthetic construct
SSSSGSSSSG

SEQ ID NO: 19 - protein, 43 aa, synthetic construct
GGEPVWLPNLNPDQLCAFIRSAEDDPSQSANLLAEAKKLNDAQ

SEQ ID NO: 20 - protein, 43 aa, synthetic construct
GGEPVYLPNLKADQLCAFMRSLEDDPSQSANLLAEAKKLNDAQ

SEQ ID NO: 21 - protein, 43 aa, synthetic construct
GGEVVMLPNLNADQWCAFFRNLEDDPSQSANLLAEAKKLNDAQ

SEQ ID NO: 22 - protein, 43 aa, synthetic construct
GGEAVYLPNLNADQWCAFFRSLEDDPSQSANLLAEAKKLNDAQ

SEQ ID NO: 23 - protein, 47 aa, synthetic construct
AGGERIVLPNLNADQLCAFIRSLEDDPSQSANLVAEAKKLNDAQAPK

SEQ ID NO: 24 - protein, 47 aa, synthetic construct
AGGERIYLPNLNADQLCAFIRSLEDDPSQSANLLAEAKKLNDAQAPK

SEQ ID NO: 25 - protein, 47 aa, synthetic construct
AGGEPVYLPNLNADQLCAFIRSLEDDPSQSANLLAEAKKLNDAQAPK

SEQ ID NO: 26 - protein, 47 aa, synthetic construct
AGGELVYLPNLNADQLCAFIRSAEDDPSQSANLLAEAKKLNDAQAPK

SEQ ID NO: 27 - protein, 47 aa, synthetic construct
AGGERVYMPNLKADQLCAFIRSAEDDPSQSANLLAEAKKLNDAQAPK

SEQ ID NO: 28 - protein, 47 aa, synthetic construct
AGGETFSLPNLNADQLCAFIRSLEDDPSQSANLVAEAKKLNDAQAPK

SEQ ID NO: 29 - skipped

SEQ ID NO: 30 - protein, 47 aa, synthetic construct
AGGERFYLPNLNPDQLCAFIRSLEDDPSQSANLIAEAKKLNDAQAPK

SEQ ID NO: 31 - protein, 47 aa, synthetic construct
AGGERFTLPNLNADQLCAFIRSLEDDPSQSANLLAEAKKLNDAQAPK

SEQ ID NO: 32 - protein, 47 aa, synthetic construct
AGGERFTLPNLNPDQICAFIRSVEDDPSQSANLLAEAKKLNDAQAPK

SEQ ID NO: 33 - protein, 47 aa, synthetic construct
AGGEEVYLPNLKADQLCAFIRSVEDDPSQSANLLAEAKKLNDAQAPK

SEQ ID NO: 34 - protein, 47 aa, synthetic construct
AGGEPVYLPNLNPDQWCAFLRSLEDDPSQSANLLAEAKKLNDAQAPK

SEQ ID NO: 35 - protein, 47 aa, synthetic construct
AGGEPVYLPNLNADQWCAFWRSLEDDPSQSANLLAEAKKLNDAQAPK

SEQ ID NO: 36 - protein, 47 aa, synthetic construct
AGGERVYYPNLNADQWCAFWRSLEDDPSQSANLLAEAKKLNDAQAPK

SEQ ID NO: 37 - protein, 47 aa, synthetic construct
AGGETVLLPNLNPDQWCAFWRSLEDDPSQSANLLAEAKKLNDAQAPK

SEQ ID NO: 38 - protein, 47 aa, synthetic construct
AGGEIVWLPNLNPDQWCAFFRSLEDDPSQSANLLAEAKKLNDAQAPK

SEQ ID NO: 39 - protein, 47 aa, synthetic construct
AGGERVYLPNLKADQLCAFFRSLEDDPSQSANLLAEAKKLNDAQAPK

SEQ ID NO: 40 - skipped

SEQ ID NO: 41 - protein, 47 aa, synthetic construct
AGGEPVWLPNLNPDQLCAFIRSAEDDPSQSANLLAEAKKLNDAQAPK

SEQ ID NO: 42 - protein, 47 aa, synthetic construct
AGGEPVYLPNLKADQLCAFMRSLEDDPSQSANLLAEAKKLNDAQAPK

SEQ ID NO: 43 - protein, 47 aa, synthetic construct
AGGEVVMLPNLNADQWCAFFRNLEDDPSQSANLLAEAKKLNDAQAPK

SEQ ID NO: 44 - protein, 47 aa, synthetic construct
AGGEAVYLPNLNADQWCAFFRSLEDDPSQSANLLAEAKKLNDAQAPK

SEQ ID NO: 45 - protein, 43 aa, synthetic construct
GXXXXXXXXXXXXXXCXFIXXXXXXXXXXAXXXXXXXXXXXXX

SEQ ID NO: 46 - protein, 43 aa, synthetic construct
XGXXVXXXXXXXXXXCXFXXXXXXXXXXXAXXLXXXXXXXXXX

SEQ ID NO: 47 - protein, 4 aa, synthetic construct
RIVL

SEQ ID NO: 48 - protein, 4 aa, synthetic construct
RIYL

SEQ ID NO: 49 - protein, 4 aa, synthetic construct
PVYL

SEQ ID NO: 50 - protein, 4 aa, synthetic construct
LVYL

SEQ ID NO: 51 - protein, 4 aa, synthetic construct
RVYM

SEQ ID NO: 52 - protein, 4 aa, synthetic construct
TFSL

SEQ ID NO: 53 - protein, 4 aa, synthetic construct
RFYL

SEQ ID NO: 54 - protein, 4 aa, synthetic construct
RFTL

SEQ ID NO: 55 - protein, 4 aa, synthetic construct
EVYL

SEQ ID NO: 56 - protein, 4 aa, synthetic construct
TVLL

SEQ ID NO: 57 - protein, 4 aa, synthetic construct
RVYL